European Patent Specification EP 3 842 522 B1, published October 15, 2025. Title: Method for generating regulatory T cells. Applicant: OSAKA UNIVERSITY. The sequence listing filed with the application follows.

SEQUENCE LISTING (4 sequences)

SEQ ID NO: 1 - DNA, 22 bp, Artificial Sequence
  primer
atttgaattggatatggtttgt

SEQ ID NO: 2 - DNA, 22 bp, Artificial Sequence
  primer
aaccttaaacccctctaacatc

SEQ ID NO: 3 - DNA, 25 bp, Artificial Sequence
  primer
ttgggttaagtttgttgtaggatag

SEQ ID NO: 4 - DNA, 25 bp, Artificial Sequence
  primer
atctaaaccctattatcacaacccc